European Patent Specification EP 3 810 175 B1, published December 25, 2024. Title: Cancer-specific T-cell Receptors. Applicant: University College Cardiff Consultants Limited. The sequence listing filed with the application follows.

SEQUENCE LISTING (86 sequences)

SEQ ID NO: 1 - protein, 17 aa, Homo sapiens
CATSDRGQGANWDEQFF

SEQ ID NO: 2 - protein, 13 aa, Homo sapiens
CASTLGGGTEAFF

SEQ ID NO: 3 - protein, 15 aa, Homo sapiens
CSARDLLAETYEQYF

SEQ ID NO: 4 - protein, 13 aa, Homo sapiens
CASSSSDTDTQYF

SEQ ID NO: 5 - protein, 18 aa, Homo sapiens
CSVEGSLGRALRANEQFF

SEQ ID NO: 6 - protein, 11 aa, Homo sapiens
CATHGGEKLFF

SEQ ID NO: 7 - protein, 14 aa, Homo sapiens
CASSYVGLGSPLHF

SEQ ID NO: 8 - protein, 11 aa, Homo sapiens
CSGQANTEAFF

SEQ ID NO: 9 - protein, 17 aa, Homo sapiens
CASSPTTGLKTRSGYTF

SEQ ID NO: 10 - protein, 12 aa, Homo sapiens
CSEGSPYNEQFF

SEQ ID NO: 11 - protein, 14 aa, Homo sapiens
CASSNGFHFNTLYF

SEQ ID NO: 12 - protein, 13 aa, Homo sapiens
CASSLGGGDTQYF

SEQ ID NO: 13 - protein, 13 aa, Homo sapiens
CASSFAGTDTQYF

SEQ ID NO: 14 - protein, 15 aa, Homo sapiens
CASSLGEGSPGELFF

SEQ ID NO: 15 - protein, 15 aa, Homo sapiens
CASSQEPNWNTEAFF

SEQ ID NO: 16 - protein, 14 aa, Homo sapiens
CASSFQGPGYGYTF

SEQ ID NO: 17 - protein, 14 aa, Homo sapiens
CSARDTTWGLEQYF

SEQ ID NO: 18 - protein, 14 aa, Homo sapiens
CATKPSGSTDTQYF

SEQ ID NO: 19 - protein, 14 aa, Homo sapiens
CSARDEGIGYEQYF

SEQ ID NO: 20 - protein, 12 aa, Homo sapiens
CASSSGPGELFF

SEQ ID NO: 21 - protein, 20 aa, Homo sapiens
CARRTLVIVRRFYSGNTIYF

SEQ ID NO: 22 - protein, 16 aa, Homo sapiens
CSARDLIGSQTYEQYF

SEQ ID NO: 23 - protein, 16 aa, Homo sapiens
CSARDPIGTESYEQYF

SEQ ID NO: 24 - protein, 14 aa, Homo sapiens
CSARDRAGRSPLHF

SEQ ID NO: 25 - protein, 14 aa, Homo sapiens
CSVEESSGIYEQYF

SEQ ID NO: 26 - protein, 15 aa, Homo sapiens
CSAREDGGQTYEQYF

SEQ ID NO: 27 - protein, 13 aa, Homo sapiens
CASSWAGPVEQYF

SEQ ID NO: 28 - protein, 13 aa, Homo sapiens
CASSSQGRAEQYF

SEQ ID NO: 29 - protein, 14 aa, Homo sapiens
CASSSRDSLYEQYF

SEQ ID NO: 30 - protein, 15 aa, Homo sapiens
CASSLGIISGQPQHF

SEQ ID NO: 31 - protein, 13 aa, Homo sapiens
CASSNTGGYTQYF

SEQ ID NO: 32 - protein, 15 aa, Homo sapiens
CASSQGLLLDNEQFF

SEQ ID NO: 33 - protein, 17 aa, Homo sapiens
CASSSPMDSGDTDTQYF

SEQ ID NO: 34 - protein, 13 aa, Homo sapiens
CASSPRSGVPQHF

SEQ ID NO: 35 - protein, 17 aa, Homo sapiens
CASSFVREEGSTDTQYF

SEQ ID NO: 36 - protein, 13 aa, Homo sapiens
CSARGTESYEQYF

SEQ ID NO: 37 - protein, 15 aa, Homo sapiens
CASWPGEGFGETQYF

SEQ ID NO: 38 - protein, 13 aa, Homo sapiens
CSGWGQGDEKLFF

SEQ ID NO: 39 - protein, 15 aa, Homo sapiens
CASSEYTSGNQPQHF

SEQ ID NO: 40 - protein, 16 aa, Homo sapiens
CSARDLWTGETYEQYF

SEQ ID NO: 41 - protein, 14 aa, Homo sapiens
CSATGLAGLGEQFF

SEQ ID NO: 42 - protein, 15 aa, Homo sapiens
CATSDLGTGVGEQFF

SEQ ID NO: 43 - protein, 13 aa, Homo sapiens
CSVGPGSTGELFF

SEQ ID NO: 44 - protein, 12 aa, Homo sapiens
CASSPTGEKLFF

SEQ ID NO: 45 - protein, 16 aa, Homo sapiens
CASSQEGGTWGDGYTF

SEQ ID NO: 46 - protein, 20 aa, Homo sapiens
CATSDLLLAGGRSSYNEQFF

SEQ ID NO: 47 - protein, 14 aa, Homo sapiens
CASSEAASGRPQTF

SEQ ID NO: 48 - protein, 19 aa, Homo sapiens
CATSDATAGTSGSLYEQYF

SEQ ID NO: 49 - protein, 14 aa, Homo sapiens
CASSLTGLGQPQHF

SEQ ID NO: 50 - protein, 14 aa, Homo sapiens
CASSPAVLSYEQYF

SEQ ID NO: 51 - protein, 15 aa, Homo sapiens
CSARESLAETYEQYF

SEQ ID NO: 52 - protein, 14 aa, Homo sapiens
CASSPGLTANVLTF

SEQ ID NO: 53 - protein, 14 aa, Homo sapiens
CASSLGLAGNEQYF

SEQ ID NO: 54 - protein, 14 aa, Homo sapiens
CASSNGFHFNTQYF

SEQ ID NO: 55 - protein, 14 aa, Homo sapiens
CASSLGILTDTQYF

SEQ ID NO: 56 - protein, 13 aa, Homo sapiens
CASSFQPVDTQYF

SEQ ID NO: 57 - protein, 13 aa, Homo sapiens
CSASEGIGQPQHF

SEQ ID NO: 58 - protein, 12 aa, Homo sapiens
CASSVSGGEQFF

SEQ ID NO: 59 - protein, 17 aa, Homo sapiens
CATSDRGQGANWDEQFF

SEQ ID NO: 60 - protein, 13 aa, Homo sapiens
CASTLGGGTEAFF

SEQ ID NO: 61 - protein, 15 aa, Homo sapiens
CSARDLLAETYEQYF

SEQ ID NO: 62 - protein, 13 aa, Homo sapiens
CASSSSDTDTQYF

SEQ ID NO: 63 - protein, 18 aa, Homo sapiens
CSVEGSLGRALRANEQFF

SEQ ID NO: 64 - protein, 11 aa, Homo sapiens
CATHGGEKLFF

SEQ ID NO: 65 - protein, 14 aa, Homo sapiens
CASSYVGLGSPLHF

SEQ ID NO: 66 - protein, 11 aa, Homo sapiens
CSGQANTEAFF

SEQ ID NO: 67 - protein, 17 aa, Homo sapiens
CASSPTTGLKTRSGYTF

SEQ ID NO: 68 - protein, 12 aa, Homo sapiens
CSEGSPYNEQFF

SEQ ID NO: 69 - protein, 14 aa, Homo sapiens
CASSNGFHFNTLYF

SEQ ID NO: 70 - protein, 13 aa, Homo sapiens
CASSLGGGDTQYF

SEQ ID NO: 71 - protein, 10 aa, Homo sapiens
EAAGIGILTV

SEQ ID NO: 72 - protein, 10 aa, Homo sapiens
LLLGIGILVL

SEQ ID NO: 73 - protein, 10 aa, Homo sapiens
NLSALGIFST

SEQ ID NO: 74 - protein, 9 aa, Homo sapiens
RLVDDFLLV

SEQ ID NO: 75 - protein, 9 aa, Homo sapiens
ALKDVEERV

SEQ ID NO: 76 - protein, 10 aa, Homo sapiens
ITSAIGVLPV

SEQ ID NO: 77 - protein, 10 aa, Homo sapiens
ITSAIGILPV

SEQ ID NO: 78 - protein, 10 aa, Homo sapiens
MTSAIGVLPV

SEQ ID NO: 79 - protein, 10 aa, Homo sapiens
QTSAIGVLPV

SEQ ID NO: 80 - protein, 10 aa, Homo sapiens
MTSAIGILPV

SEQ ID NO: 81 - protein, 10 aa, Homo sapiens
LTSAIGVLPV

SEQ ID NO: 82 - protein, 10 aa, Homo sapiens
ITSGIGVLPV

SEQ ID NO: 83 - protein, 10 aa, Homo sapiens
ITSAIGVLPI

SEQ ID NO: 84 - protein, 10 aa, Homo sapiens
QTSAIGILPV

SEQ ID NO: 85 - protein, 10 aa, Homo sapiens
ITSAIGVLFV

SEQ ID NO: 86 - protein, 10 aa, Homo sapiens
ALWGPDPAAA